European Patent Specification EP 3 878 859 B1, published November 1, 2023. Title: NOVEL OXYNTOMODULIN DERIVATIVES AND PHARMACEUTICAL COMPOSITION FOR TREATING OBESITY COMPRISING THE SAME. Applicant: HANMI SCIENCE CO., LTD. The sequence listing filed with the application follows.

SEQUENCE LISTING (56 sequences)

SEQ ID NO: 1 - protein, 37 aa, Homo sapiens
  MISC_FEATURE (1)..(37): Oxyntomodulin
HSQGTFTSDYSKYLDSRRAQDFVQWLMNTKRNRNNIA

SEQ ID NO: 2 - protein, 37 aa, Artificial Sequence
  Description of Artificial Sequence: Synthetic polypeptide construct of Oxyntomodulin derivative
  MOD_RES (1)..(1): 4-imidazoacetyl
HSQGTFTSDYSKYLDEEAVRLFIEWLMNTKRNRNNIA

SEQ ID NO: 3 - protein, 39 aa, Artificial Sequence
  Description of Artificial Sequence: Synthetic polypeptide construct of Oxyntomodulin derivative
  MOD_RES (1)..(1): 4-imidazoacetyl
HSQGTFTSDYSKYLDERRAQDFVAWLKNTGPSSGAPPPS

SEQ ID NO: 4 - protein, 39 aa, Artificial Sequence
  Description of Artificial Sequence: Synthetic polypeptide construct of Oxyntomodulin derivative
  MOD_RES (1)..(1): 4-imidazoacetyl
HGQGTFTSDYSRYLEEEAVRLFIEWLKNGGPSSGAPPPS

SEQ ID NO: 5 - protein, 39 aa, Artificial Sequence
  Description of Artificial Sequence: Synthetic polypeptide construct of Oxyntomodulin derivative
  MOD_RES (1)..(1): 4-imidazoacetyl
HGQGTFTSDYSRQMEEEAVRLFIEWLKNGGPSSGAPPPS

SEQ ID NO: 6 - protein, 42 aa, Artificial Sequence
  Description of Artificial Sequence: Synthetic polypeptide construct of Oxyntomodulin derivative
  MOD_RES (1)..(1): 4-imidazoacetyl
HGEGTFTSDLSRQMEEEAVRLFIEWAAHSQGTFTSDYSKYLD

SEQ ID NO: 7 - protein, 30 aa, Artificial Sequence
  Description of Artificial Sequence: Synthetic polypeptide construct of Oxyntomodulin derivative
  MOD_RES (1)..(1): 4-imidazoacetyl
HSQGTFTSDYSRYLDEEAVRLFIEWLMNTK

SEQ ID NO: 8 - protein, 29 aa, Artificial Sequence
  Description of Artificial Sequence: Synthetic peptide construct of Oxyntomodulin derivative
  MOD_RES (1)..(1): 4-imidazoacetyl
HSQGTFTSDLSRQLEEEAVRLFIEWLMNK

SEQ ID NO: 9 - protein, 37 aa, Artificial Sequence
  Description of Artificial Sequence: Synthetic polypeptide construct of Oxyntomodulin derivative
  MOD_RES (1)..(1): 4-imidazoacetyl
  MOD_RES (20)..(20): Alpha-methyl-glutamic acid
HGQGTFTSDYSRYLDEEAVELFIEWLMNTKRNRNNIA

SEQ ID NO: 10 - protein, 40 aa, Artificial Sequence
  Description of Artificial Sequence: Synthetic polypeptide construct of Oxyntomodulin derivative
  MOD_RES (1)..(1): 4-imidazoacetyl
HSQGTFTSDYSRQMEEEAVRLFIEWLMNGGPSSGAPPPSK

SEQ ID NO: 11 - protein, 43 aa, Artificial Sequence
  Description of Artificial Sequence: Synthetic polypeptide construct of Oxyntomodulin derivative
  MOD_RES (1)..(1): 4-imidazoacetyl
HGEGTFTSDLSRQMEEEAVRLFIEWAAHSQGTFTSDYSRYLDK

SEQ ID NO: 12 - protein, 38 aa, Artificial Sequence
  Description of Artificial Sequence: Synthetic polypeptide construct of Oxyntomodulin derivative
  MOD_RES (1)..(1): 4-imidazoacetyl
HSQGTFTSDYSRYLDGGGHGEGTFTSDLSKQMEEEAVK

SEQ ID NO: 13 - protein, 30 aa, Artificial Sequence
  Description of Artificial Sequence: Synthetic polypeptide construct of Oxyntomodulin derivative
  MOD_RES (1)..(1): 4-imidazoacetyl
  MOD_RES (16)..(16): Alpha-methyl-glutamic acid
  MOD_RES (20)..(20): Alpha-methyl-glutamic acid
HSQGTFTSDYSRYLDEEAVELFIEWLMNTK

SEQ ID NO: 14 - protein, 37 aa, Artificial Sequence; identical to SEQ ID NO: 9
  Description of Artificial Sequence: Synthetic polypeptide construct of Oxyntomodulin derivative
  MOD_RES (1)..(1): 4-imidazoacetyl
  MOD_RES (20)..(20): Alpha-methyl-glutamic acid
  MOD_RES (24)..(24): Alpha-methyl-glutamic acid

SEQ ID NO: 15 - protein, 37 aa, Artificial Sequence
  Description of Artificial Sequence: Synthetic polypeptide construct of Oxyntomodulin derivative
  MOD_RES (1)..(1): 4-imidazoacetyl
  MOD_RES (24)..(24): Alpha-methyl-glutamic acid
HGQGTFTSDYSRYLDEEAVRLFIEWLMNTKRNRNNIA

SEQ ID NO: 16 - protein, 34 aa, Artificial Sequence
  Description of Artificial Sequence: Synthetic polypeptide construct of Oxyntomodulin derivative
  MOD_RES (1)..(1): 4-imidazoacetyl
HSQGTFTSDLSRQLEGGGHSQGTFTSDLSRQLEK

SEQ ID NO: 17 - protein, 37 aa, Artificial Sequence
  Description of Artificial Sequence: Synthetic polypeptide construct of Oxyntomodulin derivative
  MOD_RES (1)..(1): 4-imidazoacetyl
HSQGTFTSDYSRYLDEEAVRLFIEWIRNTKRNRNNIA

SEQ ID NO: 18 - protein, 40 aa, Artificial Sequence
  Description of Artificial Sequence: Synthetic polypeptide construct of Oxyntomodulin derivative
  MOD_RES (1)..(1): 4-imidazoacetyl
HSQGTFTSDYSRYLDEEAVRLFIEWIRNGGPSSGAPPPSK

SEQ ID NO: 19 - protein, 37 aa, Artificial Sequence
  Description of Artificial Sequence: Synthetic polypeptide construct of Oxyntomodulin derivative
  MOD_RES (1)..(1): 4-imidazoacetyl
  MISC_FEATURE (16)..(20): Ring formation between residues
HSQGTFTSDYSRYLDEEAVKLFIEWIRNTKRNRNNIA

SEQ ID NO: 20 - protein, 40 aa, Artificial Sequence
  Description of Artificial Sequence: Synthetic polypeptide construct of Oxyntomodulin derivative
  MOD_RES (1)..(1): 4-imidazoacetyl
  MISC_FEATURE (16)..(20): Ring formation between residues
HSQGTFTSDYSRYLDEEAVKLFIEWIRNGGPSSGAPPPSK

SEQ ID NO: 21 - protein, 37 aa, Artificial Sequence
  Description of Artificial Sequence: Synthetic polypeptide construct of Oxyntomodulin derivative
  MOD_RES (1)..(1): 4-imidazoacetyl
HSQGTFTSDYSRQLEEEAVRLFIEWVRNTKRNRNNIA

SEQ ID NO: 22 - protein, 30 aa, Artificial Sequence
  Description of Artificial Sequence: Synthetic polypeptide construct of Oxyntomodulin derivative
  MOD_RES (1)..(1): Desamino-histidyl
  MISC_FEATURE (16)..(20): Ring formation between residues
HSQGTFTSDYSKYLDEKRAKEFVQWLMNTK

SEQ ID NO: 23 - protein, 29 aa, Artificial Sequence
  Description of Artificial Sequence: Synthetic peptide construct of Oxyntomodulin derivative
  MOD_RES (2)..(2): Aib
HXQGTFTSDYSKYLDEKRAKEFVCWLMNT

SEQ ID NO: 24 - protein, 30 aa, Artificial Sequence
  Description of Artificial Sequence: Synthetic polypeptide construct of Oxyntomodulin derivative
  MOD_RES (2)..(2): Aib
HXQGTFTSDYSKYLDEKRAKEFVQWLMNTC

SEQ ID NO: 25 - protein, 30 aa, Artificial Sequence; identical to SEQ ID NO: 24
  Description of Artificial Sequence: Synthetic polypeptide construct of Oxyntomodulin derivative
  MOD_RES (2)..(2): Aib
  MISC_FEATURE (16)..(20): Ring formation between residues

SEQ ID NO: 26 - protein, 30 aa, Artificial Sequence; identical to SEQ ID NO: 24
  Description of Artificial Sequence: Synthetic polypeptide construct of Oxyntomodulin derivative
  MOD_RES (2)..(2): Aib
  MOD_RES (12)..(16): Ring formation between residues

SEQ ID NO: 27 - protein, 29 aa, Artificial Sequence
  Description of Artificial Sequence: Synthetic peptide construct of Oxyntomodulin derivative
  MOD_RES (2)..(2): Aib
  MISC_FEATURE (16)..(20): Ring formation between residues
HXQGTFTSDYSKYLDEQAAKEFICWLMNT

SEQ ID NO: 28 - protein, 29 aa, Artificial Sequence
  Description of Artificial Sequence: Synthetic peptide construct of Oxyntomodulin derivative
  MOD_RES (2)..(2): Aib
HXQGTFTSDYSKYLDEKRAKEFVQWLMNT

SEQ ID NO: 29 - protein, 30 aa, Artificial Sequence; identical to SEQ ID NO: 24
  Description of Artificial Sequence: Synthetic polypeptide oxyntomodulin derivative
  MOD_RES (1)..(1): 4-imidazoacetyl
  MOD_RES (2)..(2): Aib
  MISC_FEATURE (16)..(20): Ring formation between residues

SEQ ID NO: 30 - protein, 30 aa, Artificial Sequence
  Description of Artificial Sequence: Synthetic polypeptide oxyntomodulin derivative
  MOD_RES (2)..(2): Aib
  MISC_FEATURE (16)..(20): Ring formation between residues
HXQGTFTSDYAKYLDEKRAKEFVQWLMNTC

SEQ ID NO: 31 - protein, 30 aa, Artificial Sequence
  Description of Artificial Sequence: Synthetic polypeptide oxyntomodulin derivative
  MOD_RES (2)..(2): Aib
  MISC_FEATURE (16)..(20): Ring formation between residues
YXQGTFTSDYSKYLDEKRAKEFVQWLMNTC

SEQ ID NO: 32 - protein, 8 aa, Artificial Sequence
  Description of Artificial Sequence: Synthetic peptide construct of group R2
KRNRNNIA

SEQ ID NO: 33 - protein, 10 aa, Artificial Sequence
  Description of Artificial Sequence: Synthetic peptide construct of group R2
GPSSGAPPPS

SEQ ID NO: 34 - protein, 11 aa, Artificial Sequence
  Description of Artificial Sequence: Synthetic peptide construct of group R2
GPSSGAPPPSK

SEQ ID NO: 35 - protein, 15 aa, Artificial Sequence
  Description of Artificial Sequence: Synthetic peptide construct of group R2
HSQGTFTSDYSKYLD

SEQ ID NO: 36 - protein, 16 aa, Artificial Sequence
  Description of Artificial Sequence: Synthetic peptide construct of group R2
HSQGTFTSDYSRYLDK

SEQ ID NO: 37 - protein, 20 aa, Artificial Sequence
  Description of Artificial Sequence: Synthetic peptide construct of group R2
HGEGTFTSDLSKQMEEEAVK

SEQ ID NO: 38 - protein, 28 aa, Artificial Sequence
  Description of Artificial Sequence: Synthetic peptide construct of group A or B
SQGTFTSDYSKYLDSRRAQDFVQWLMNT

SEQ ID NO: 39 - protein, 28 aa, Artificial Sequence
  Description of Artificial Sequence: Synthetic peptide construct of group A or B
SQGTFTSDYSKYLDEEAVRLFIEWLMNT

SEQ ID NO: 40 - protein, 28 aa, Artificial Sequence
  Description of Artificial Sequence: Synthetic peptide construct of group A or B
SQGTFTSDYSKYLDERRAQDFVAWLKNT

SEQ ID NO: 41 - protein, 28 aa, Artificial Sequence
  Description of Artificial Sequence: Synthetic peptide construct of group A or B
GQGTFTSDYSRYLEEEAVRLFIEWLKNG

SEQ ID NO: 42 - protein, 28 aa, Artificial Sequence
  Description of Artificial Sequence: Synthetic peptide construct of group A or B
GQGTFTSDYSRQMEEEAVRLFIEWLKNG

SEQ ID NO: 43 - protein, 26 aa, Artificial Sequence
  Description of Artificial Sequence: Synthetic peptide construct of group A or B
GEGTFTSDLSRQMEEEAVRLFIEWAA

SEQ ID NO: 44 - protein, 28 aa, Artificial Sequence
  Description of Artificial Sequence: Synthetic peptide construct of group A or B
SQGTFTSDYSRQMEEEAVRLFIEWLMNG

SEQ ID NO: 45 - protein, 24 aa, Artificial Sequence
  Description of Artificial Sequence: Synthetic peptide construct of group B
GEGTFTSDLSRQMEEEAVRLFIEW

SEQ ID NO: 46 - protein, 14 aa, Artificial Sequence
  Description of Artificial Sequence: Synthetic peptide construct of group B
SQGTFTSDYSRYLD

SEQ ID NO: 47 - DNA, 30 bp, Artificial Sequence
  Description of Artificial Sequence: Synthetic primer
cccggcccccgcggccgctattcgaaatac

SEQ ID NO: 48 - DNA, 33 bp, Artificial Sequence
  Description of Artificial Sequence: Synthetic primer
gaacggtccggaggacgtcgactcttaagatag

SEQ ID NO: 49 - DNA, 34 bp, Artificial Sequence
  Description of Artificial Sequence: Synthetic primer
cagcgacaccgaccgtccccccgtacttaaggcc

SEQ ID NO: 50 - DNA, 32 bp, Artificial Sequence
  Description of Artificial Sequence: Synthetic primer
ctaaccgactctcggggaagactgagctcgcc

SEQ ID NO: 51 - protein, 60 aa, Artificial Sequence
  Description of Artificial Sequence: Synthetic polypeptide
  MOD_RES (1)..(1): Histidine, desamino-histidyl, dimethyl-histidyl (N-dimethyl- histidyl), beta-hydroxyimidazopropionyl, 4-imidazoacetyl, beta-carboxy imidazopropionyl or tyrosine
  MOD_RES (2)..(2): Aib(aminosiobutyric acid), d-alanine, glycine, Sar(N-methylglycine), serine or d-serine
  MOD_RES (3)..(3): Glutamic acid or glutamine
  MOD_RES (10)..(10): Leucine or tyrosine
  MOD_RES (11)..(11): Serine or alanine
  MOD_RES (12)..(12): Lysine or arginine
  MOD_RES (13)..(13): Glutamine or tyrosine
  MOD_RES (14)..(14): Leucine or methionine
  MOD_RES (15)..(15): Aspartic acid or glutamic acid
  MOD_RES (16)..(16): Glutamic acid, serine, alpha-methyl-glutamic acid or not present
  MOD_RES (17)..(17): Glutamine, glutamic acid, lysine, arginine, serine or not present
  MOD_RES (18)..(18): Alanine, arginine, valine or not present
  MOD_RES (19)..(19): Alanine, arginine, serine, valine or not present
  MOD_RES (20)..(20): Lysine, glutamine, arginine, alpha-methyl-glutamic acid or not present
  MOD_RES (21)..(21): Aspartic acid, glutamic acid, leucine or not present
  MISC_FEATURE (22)..(22): May or may not be present
  MOD_RES (23)..(23): Isoleucine, valine or not present
  MOD_RES (24)..(24): Alanine, cysteine, glutamic acid, lysine, glutamine, alpha-methyl-glutamic acid or not present
  MISC_FEATURE (25)..(25): May or may not be present
  MOD_RES (26)..(26): Alanine, isoleucine, leucine, serine, valine or not present
  MOD_RES (27)..(27): Alanine, lysine, methionine, glutamine, arginine or not present
  MISC_FEATURE (28)..(28): May or may not be present
  MOD_RES (29)..(29): Alanine, glycine, threonine or not present
  MOD_RES (30)..(30): Cysteine, lysine or not present
  MOD_RES (31)..(40): Alanine, glycine, serine or not present
  MISC_FEATURE (31)..(40): This region may encompass 2 to 10 amino acids, wherein some positions may be absent
  MISC_FEATURE (41)..(60): This region may encompass 8 to 20 amino acids including "KRNRNNIA" or "GPSSGAPPPS" or "GPSSGAPPPSK" or "HSQGTFTSDYSKYLD" or "HSQGTFTSDYSRYLDK" or "HGEGTFTSDLSKQMEEEAVK," wherein some or all positions may be absent
  See specification as filed for detailed description of substitutions and preferred embodiments
XXXGTFTSDXXXXXXXXXXXXFXXWXXNXXXXXXXXXXXXXXXXXXXXXXXXXXXXXXXX

SEQ ID NO: 52 - protein, 40 aa, Artificial Sequence
  Description of Artificial Sequence: Synthetic polypeptide
  MOD_RES (1)..(1): Histidine, desamino-histidyl, dimethyl-histidyl (N-dimethyl- histidyl), beta-hydroxyimidazopropionyl, 4-imidazoacetyl, beta-carboxy imidazopropionyl or tyrosine
  MISC_FEATURE (2)..(29): This region may encompass 26 to 28 amino acids including "SQGTFTSDYSKYLDSRRAQDFVQWLMNT" or "SQGTFTSDYSKYLDEEAVRLFIEWLMNT" or "SQGTFTSDYSKYLDERRAQDFVAWLKNT" or "GQGTFTSDYSRYLEEEAVRLFIEWLKNG" or "GQGTFTSDYSRQMEEEAVRLFIEWLKNG"
  MISC_FEATURE (2)..(29): Continued from above; or "GEGTFTSDLSRQMEEEAVRLFIEWAA" or "SQGTFTSDYSRQMEEEAVRLFIEWLMNG," wherein some positions may be absent
  MISC_FEATURE (30)..(40): This region may encompass 8 to 11 amino acids including "KRNRNNIA" or "GPSSGAPPPS" or "GPSSGAPPPSK," wherein some positions may be absent
  See specification as filed for detailed description of substitutions and preferred embodiments
XXXXXXXXXXXXXXXXXXXXXXXXXXXXXXXXXXXXXXXX

SEQ ID NO: 53 - protein, 59 aa, Artificial Sequence
  Description of Artificial Sequence: Synthetic polypeptide
  MOD_RES (1)..(1): Histidine, desamino-histidyl, dimethyl-histidyl (N-dimethyl- histidyl), beta-hydroxyimidazopropionyl, 4-imidazoacetyl, beta-carboxy imidazopropionyl or tyrosine
  MISC_FEATURE (2)..(29): This region may encompass 14 to 28 amino acids including "SQGTFTSDYSKYLDSRRAQDFVQWLMNT" or "SQGTFTSDYSKYLDEEAVRLFIEWLMNT" or "SQGTFTSDYSKYLDERRAQDFVAWLKNT" or "GQGTFTSDYSRYLEEEAVRLFIEWLKNG" or "GQGTFTSDYSRQMEEEAVRLFIEWLKNG"
  MISC_FEATURE (2)..(29): Continued from above; or "GEGTFTSDLSRQMEEEAVRLFIEWAA" or "SQGTFTSDYSRQMEEEAVRLFIEWLMNG" or "GEGTFTSDLSRQMEEEAVRLFIEW" or "SQGTFTSDYSRYLD," wherein some positions may be absent
  MOD_RES (30)..(39): Alanine, glycine, serine or not present
  MISC_FEATURE (30)..(39): This region may encompass 2 to 10 amino acids, wherein some positions may be absent
  MISC_FEATURE (40)..(59): This region may encompass 15 to 20 amino acids including "HSQGTFTSDYSKYLD" or "HSQGTFTSDYSRYLDK" or "HGEGTFTSDLSKQMEEEAVK," wherein some positions may be absent
  See specification as filed for detailed description of substitutions and preferred embodiments
XXXXXXXXXXXXXXXXXXXXXXXXXXXXXXXXXXXXXXXXXXXXXXXXXXXXXXXXXXX

SEQ ID NO: 54 - protein, 40 aa, Artificial Sequence
  Description of Artificial Sequence: Synthetic polypeptide
  MOD_RES (1)..(1): Histidine, desamino-histidyl, dimethyl-histidyl (N-dimethyl- histidyl), beta-hydroxyimidazopropionyl, 4-imidazoacetyl, beta-carboxy imidazopropionyl or tyrosine
  MOD_RES (16)..(16): Serine, glutamic acid or arginine
  MOD_RES (17)..(17): Arginine, glutamic acid or serine
  MOD_RES (18)..(18): Arginine, alanine or valine
  MOD_RES (19)..(19): Arginine, valine or serine
  MOD_RES (20)..(20): Glutamine, arginine or lysine
  MOD_RES (26)..(26): Isoleucine, valine or serine
  MOD_RES (27)..(27): Methionine, arginine or glutamine
  MOD_RES (29)..(29): Threonine, glycine or alanine
  MISC_FEATURE (30)..(40): This region may encompass 8 to 11 amino acids including "KRNRNNIA" or "GPSSGAPPPS" or "GPSSGAPPPSK," wherein some positions may be absent
  See specification as filed for detailed description of substitutions and preferred embodiments
XSQGTFTSDYSKYLDXXXXXLFVQWXXNXXXXXXXXXXXX

SEQ ID NO: 55 - protein, 41 aa, Artificial Sequence
  Description of Artificial Sequence: Synthetic polypeptide
  MOD_RES (1)..(1): Histidine, desamino-histidyl, dimethyl-histidyl (N-dimethyl- histidyl), beta-hydroxyimidazopropionyl, 4-imidazoacetyl, beta-carboxy imidazopropionyl or tyrosine
  MOD_RES (2)..(2): Serine, Aib, Sar, d-alanine or d-serine
  MOD_RES (16)..(16): Serine or glutamic acid
  MOD_RES (17)..(17): Arginine or lysine
  MOD_RES (20)..(20): Glutamine or lysine
  MOD_RES (21)..(21): Aspartic acid or glutamic acid
  MOD_RES (24)..(24): Glutamine, cysteine or lysine
  MOD_RES (30)..(30): Cysteine, lysine or not present
  MISC_FEATURE (31)..(41): This region may encompass 8 to 11 amino acids including "KRNRNNIA" or "GPSSGAPPPS" or "GPSSGAPPPSK," wherein some or all positions may be absent
  See specification as filed for detailed description of substitutions and preferred embodiments
XXQGTFTSDYSKYLDXXRAXXFVXWLMNTXXXXXXXXXXXX

SEQ ID NO: 56 - protein, 60 aa, Artificial Sequence
  Description of Artificial Sequence: Synthetic polypeptide
  MOD_RES (1)..(1): Histidine, desamino-histidyl, 4-imidazoacetyl or tyrosine
  MOD_RES (2)..(2): Aib(aminosiobutyric acid), glycine or serine
  MOD_RES (3)..(3): Glutamic acid or glutamine
  MOD_RES (10)..(10): Leucine or tyrosine
  MOD_RES (11)..(11): Serine or alanine
  MOD_RES (12)..(12): Lysine or arginine
  MOD_RES (13)..(13): Glutamine or tyrosine
  MOD_RES (14)..(14): Leucine or methionine
  MOD_RES (15)..(15): Aspartic acid or glutamic acid
  MOD_RES (16)..(16): Glutamic acid, alpha-methyl-glutamic acid or not present
  MOD_RES (17)..(17): Glutamine, glutamic acid, lysine, arginine or not present
  MOD_RES (18)..(18): Alanine, arginine or not present
  MOD_RES (19)..(19): Alanine, valine or not present
  MOD_RES (20)..(20): Lysine, glutamine, arginine, alpha-methyl-glutamic acid or not present
  MOD_RES (21)..(21): Aspartic acid, glutamic acid, leucine or not present
  MISC_FEATURE (22)..(22): May or may not be present
  MOD_RES (23)..(23): Isoleucine, valine or not present
  MOD_RES (24)..(24): Alanine, cysteine, glutamic acid, glutamine, alpha-methyl-glutamic acid or not present
  MISC_FEATURE (25)..(25): May or may not be present
  MOD_RES (26)..(26): Alanine, isoleucine, leucine, valine or not present
  MOD_RES (27)..(27): Alanine, lysine, methionine, arginine or not present
  MISC_FEATURE (28)..(29): May or may not be present
  MOD_RES (30)..(30): Cysteine, lysine or not present
  MISC_FEATURE (31)..(40): This region may encompass 2 to 10 residues, wherein some positions may not be present
  MISC_FEATURE (41)..(60): This region may encompass 8 to 20 amino acids including "KRNRNNIA" or "GPSSGAPPPS" or "GPSSGAPPPSK" or "HSQGTFTSDYSKYLD" or "HSQGTFTSDYSRYLDK" or "HGEGTFTSDLSKQMEEEAVK," wherein some or all positions may be absent
  See specification as filed for detailed description of substitutions and preferred embodiments
XXXGTFTSDXXXXXXXXXXXXFXXWXXNTXGGGGGGGGGGXXXXXXXXXXXXXXXXXXXX